European Patent Specification EP 3 116 542 B1, published July 30, 2025. Title: Reducing systemic regulatory T cell levels or activity for treatment of DISEASE and injury of the CNS. Applicant: Yeda Research and Development Co. Ltd. Eisenbach-Schwartz, Michal Baruch , Kuti Rosenzweig, Neta. The sequence listing filed with the application follows.

SEQUENCE LISTING (56 sequences)

SEQ ID NO: 1 - protein, 15 aa, Artificial Sequence
  Synthetic
AAAYAAAAAAKAAAA

SEQ ID NO: 2 - protein, 15 aa, Artificial Sequence
  Synthetic
AEKYAAAAAAKAAAA

SEQ ID NO: 3 - protein, 15 aa, Artificial Sequence
  Synthetic
AKEYAAAAAAKAAAA

SEQ ID NO: 4 - protein, 15 aa, Artificial Sequence
  Synthetic
AKKYAAAAAAKAAAA

SEQ ID NO: 5 - protein, 15 aa, Artificial Sequence
  Synthetic
AEAYAAAAAAKAAAA

SEQ ID NO: 6 - protein, 15 aa, Artificial Sequence
  Synthetic
KEAYAAAAAAKAAAA

SEQ ID NO: 7 - protein, 15 aa, Artificial Sequence
  Synthetic
AEEYAAAAAAKAAAA

SEQ ID NO: 8 - protein, 15 aa, Artificial Sequence
  Synthetic
AAEYAAAAAAKAAAA

SEQ ID NO: 9 - protein, 15 aa, Artificial Sequence
  Synthetic
EKAYAAAAAAKAAAA

SEQ ID NO: 10 - protein, 15 aa, Artificial Sequence
  Synthetic
AAKYEAAAAAKAAAA

SEQ ID NO: 11 - protein, 15 aa, Artificial Sequence
  Synthetic
AAKYAEAAAAKAAAA

SEQ ID NO: 12 - protein, 15 aa, Artificial Sequence
  Synthetic
EAAYAAAAAAKAAAA

SEQ ID NO: 13 - protein, 15 aa, Artificial Sequence
  Synthetic
EKKYAAAAAAKAAAA

SEQ ID NO: 14 - protein, 15 aa, Artificial Sequence
  Synthetic
EAKYAAAAAAKAAAA

SEQ ID NO: 15 - protein, 15 aa, Artificial Sequence
  Synthetic
AEKYAAAAAAAAAAA

SEQ ID NO: 16 - protein, 15 aa, Artificial Sequence
  Synthetic
AKEYAAAAAAAAAAA

SEQ ID NO: 17 - protein, 15 aa, Artificial Sequence
  Synthetic
AKKYEAAAAAAAAAA

SEQ ID NO: 18 - protein, 15 aa, Artificial Sequence
  Synthetic
AKKYAEAAAAAAAAA

SEQ ID NO: 19 - protein, 15 aa, Artificial Sequence
  Synthetic
AEAYKAAAAAAAAAA

SEQ ID NO: 20 - protein, 15 aa, Artificial Sequence
  Synthetic
KEAYAAAAAAAAAAA

SEQ ID NO: 21 - protein, 15 aa, Artificial Sequence
  Synthetic
AEEYKAAAAAAAAAA

SEQ ID NO: 22 - protein, 15 aa, Artificial Sequence
  Synthetic
AAEYKAAAAAAAAAA

SEQ ID NO: 23 - protein, 15 aa, Artificial Sequence
  Synthetic
EKAYAAAAAAAAAAA

SEQ ID NO: 24 - protein, 15 aa, Artificial Sequence
  Synthetic
AAKYEAAAAAAAAAA

SEQ ID NO: 25 - protein, 15 aa, Artificial Sequence
  Synthetic
AAKYAEAAAAAAAAA

SEQ ID NO: 26 - protein, 15 aa, Artificial Sequence
  Synthetic
EKKYAAAAAAAAAAA

SEQ ID NO: 27 - protein, 15 aa, Artificial Sequence
  Synthetic
EAKYAAAAAAAAAAA

SEQ ID NO: 28 - protein, 15 aa, Artificial Sequence
  Synthetic
AEYAKAAAAAAAAAA

SEQ ID NO: 29 - protein, 15 aa, Artificial Sequence
  Synthetic
AEKAYAAAAAAAAAA

SEQ ID NO: 30 - protein, 15 aa, Artificial Sequence
  Synthetic
EKYAAAAAAAAAAAA

SEQ ID NO: 31 - protein, 15 aa, Artificial Sequence
  Synthetic
AYKAEAAAAAAAAAA

SEQ ID NO: 32 - protein, 15 aa, Artificial Sequence
  Synthetic
AKYAEAAAAAAAAAA

SEQ ID NO: 33 - DNA, 24 bp, Artificial Sequence
  Synthetic
agcatacaggtcctggcatcttgt

SEQ ID NO: 34 - DNA, 24 bp, Artificial Sequence
  Synthetic
caaagaccacatgcttgccatcca

SEQ ID NO: 35 - DNA, 24 bp, Artificial Sequence
  Synthetic
agatcacattcacggtgctggcta

SEQ ID NO: 36 - DNA, 24 bp, Artificial Sequence
  Synthetic
agctttgggatggtagctggaaga

SEQ ID NO: 37 - DNA, 24 bp, Artificial Sequence
  Synthetic
tgtgaagggattaacgaggctgga

SEQ ID NO: 38 - DNA, 24 bp, Artificial Sequence
  Synthetic
ccatgtttcgggcacatttccaca

SEQ ID NO: 39 - DNA, 21 bp, Artificial Sequence
  Synthetic
aactgcatccatatcgatgac

SEQ ID NO: 40 - DNA, 19 bp, Artificial Sequence
  Synthetic
gtggcaatgatctcaacac

SEQ ID NO: 41 - DNA, 18 bp, Artificial Sequence
  Synthetic
catccacgtgttggctca

SEQ ID NO: 42 - DNA, 23 bp, Artificial Sequence
  Synthetic
gatcatcttgctggtgaatgagt

SEQ ID NO: 43 - DNA, 20 bp, Artificial Sequence
  Synthetic
gcctcttctcattcctgctt

SEQ ID NO: 44 - DNA, 20 bp, Artificial Sequence
  Synthetic
ctcctccacttggtggtttg

SEQ ID NO: 45 - DNA, 21 bp, Artificial Sequence
  Synthetic
ccaaaagatgaagggctgctt

SEQ ID NO: 46 - DNA, 20 bp, Artificial Sequence
  Synthetic
tgctgctgcgagatttgaag

SEQ ID NO: 47 - DNA, 20 bp, Artificial Sequence
  Synthetic
gaagttcaacatcaagagca

SEQ ID NO: 48 - DNA, 19 bp, Artificial Sequence
  Synthetic
catagtccctttggtccag

SEQ ID NO: 49 - DNA, 24 bp, Artificial Sequence
  Synthetic
tgaattccctgggtgagaagctga

SEQ ID NO: 50 - DNA, 24 bp, Artificial Sequence
  Synthetic
tggccttgtagacaccttggtctt

SEQ ID NO: 51 - DNA, 24 bp, Artificial Sequence
  Synthetic
aattgctgccttcgccctctttac

SEQ ID NO: 52 - DNA, 24 bp, Artificial Sequence
  Synthetic
tgtacaggctgaggactttggtgt

SEQ ID NO: 53 - DNA, 19 bp, Artificial Sequence
  Synthetic
ccggaccagagaccctttg

SEQ ID NO: 54 - DNA, 23 bp, Artificial Sequence
  Synthetic
cctgtgggcttgttgaagtaaaa

SEQ ID NO: 55 - DNA, 24 bp, Artificial Sequence
  Synthetic
gatgctcagcagtcaagtgccttt

SEQ ID NO: 56 - DNA, 24 bp, Artificial Sequence
  Synthetic
gacatgtttgcggcatccaggtaa